European Patent Application EP 4 628 095 A1, published October 8, 2025. Title: Fusion protein and a granulated antigen containing same. Applicant: XIAMEN University. Application WO. The sequence listing filed with the application follows.

SEQUENCE LISTING (143 sequences)

SEQ ID NO: 1 - protein, 223 aa, synthetic construct
RVQPTESIVRFPNITNLCPFGEVFNATRFASVYAWNRKRISNCVADYSVLYNSASFSTFKCYGVSPTKLNDLCFTNVYADSFVIRGDEVRQIAPGQTGKIADYNYKLPDDFTGCVIAWNSNNLDSKVGGNYNYLYRLFRKSNLKPFERDISTEIYQAGSTPCNGVEGFNCYFPLQSYGFQPTNGVGYQPYRVVVLSFELLHAPATVCGPKKSTNLVKNKCVNF

SEQ ID NO: 2 - protein, 223 aa, synthetic construct
RVQPTESIVRFPNITNLCPFGEVFNATRFASVYAWNRKRISNCVADYSVLYNSASFSTFKCYGVSPTKLNDLCFTNVYADSFVIRGDEVRQIAPGQTGKIADYNYKLPDDFTGCVIAWNSNNLDSKVGGNYNYLYRLFRKSNLKPFERDISTEIYQAGSTPCNGVEGFNCYFPLQSYGFQPTYGVGYQPYRVVVLSFELLHAPATVCGPKKSTNLVKNKCVNF

SEQ ID NO: 3 - protein, 223 aa, synthetic construct
RVQPTESIVRFPNITNLCPFGEVFNATRFASVYAWNRKRISNCVADYSVLYNSASFSTFKCYGVSPTKLNDLCFTNVYADSFVIRGDEVRQIAPGQTGNIADYNYKLPDDFTGCVIAWNSNNLDSKVGGNYNYLYRLFRKSNLKPFERDISTEIYQAGSTPCNGVKGFNCYFPLQSYGFQPTYGVGYQPYRVVVLSFELLHAPATVCGPKKSTNLVKNKCVNF

SEQ ID NO: 4 - protein, 223 aa, synthetic construct
RVQPTESIVRFPNITNLCPFGEVFNATRFASVYAWNRKRISNCVADYSVLYNSASFSTFKCYGVSPTKLNDLCFTNVYADSFVIRGDEVRQIAPGQTGTIADYNYKLPDDFTGCVIAWNSNNLDSKVGGNYNYLYRLFRKSNLKPFERDISTEIYQAGSTPCNGVKGFNCYFPLQSYGFQPTYGVGYQPYRVVVLSFELLHAPATVCGPKKSTNLVKNKCVNF

SEQ ID NO: 5 - protein, 223 aa, synthetic construct
RVQPTESIVRFPNITNLCPFGEVFNATRFASVYAWNRKRISNCVADYSVLYNSASFSTFKCYGVSPTKLNDLCFTNVYADSFVIRGDEVRQIAPGQTGKIADYNYKLPDDFTGCVIAWNSNNLDSKVGGNYNYRYRLFRKSNLKPFERDISTEIYQAGSKPCNGVEGFNCYFPLQSYGFQPTNGVGYQPYRVVVLSFELLHAPATVCGPKKSTNLVKNKCVNF

SEQ ID NO: 6 - protein, 223 aa, synthetic construct
RVQPTESIVRFPNITNLCPFDEVFNATRFASVYAWNRKRISNCVADYSVLYNFAPFFAFKCYGVSPTKLNDLCFTNVYADSFVIRGNEVSQIAPGQTGNIADYNYKLPDDFTGCVIAWNSNKLDSKVGGNYNYLYRLFRKSNLKPFERDISTEIYQAGNKPCNGVAGFNCYFPLRSYGFRPTYGVGHQPYRVVVLSFELLHAPATVCGPKKSTNLVKNKCVNF

SEQ ID NO: 7 - protein, 223 aa, synthetic construct
RVQPTESIVRFPNITNLCPFDEVFNATRFASVYAWNRKRISNCVADYSVLYNFAPFFAFKCYGVSPTKLNDLCFTNVYADSFVIRGNEVSQIAPGQTGTIADYNYKLPDDFTGCVIAWNSNKLDSKVGGNYNYRYRLFRKSNLKPFERDISTEIYQAGNKPCNGVKGVNCYFPLQSYGFRPTYGVGHQPYRVVVLSFELLHAPATVCGPKKSTNLVKNKCVNF

SEQ ID NO: 8 - protein, 223 aa, synthetic construct; identical to SEQ ID NO: 7

SEQ ID NO: 9 - protein, 660 aa, synthetic construct
MRPRPILLLLLMFLPMLPAPPPGQPSGRRRGRRSGGSGGGFWGDRVDSQPFAIPYIHPTNPFAPDVTAAAGAGPRVRQPARPLGSAWRDQAQRPAAASRRRPTTAGAAPLTAVAPAHDTPPVPDVDSRGAILRRQYNLSTSPLTSSVATGTNLVLYAAPLSPLLPLQDGTNTHIMATEASNYAQYRVARATIRYRPLVPNAVGGYAISISFWPQTTTTPTSVDMNSITSTDVRILVQPGIASELVIPSERLHYRNQGWRSVETSGVAEEEATSGLVMLCIHGSPVNSYTNTPYTGALGLLDFALELEFRNLTPGNTNTRVSRYSSTARHRLRRGADGTAELTTTAATRFMKDLYFTSTNGVGEIGRGIALTLFNLADTLLGGLPTELISSAGGQLFYSRPVVSANGEPTVKLYTSVENAQQDKGIAIPHDIDLGESRVVIQDYDNQHEQDRPTPSPAPSRPFSVLRANDVLWLSLTAAEYDQSTYGSSTGPVYVSDSVTLVNVATGAQAVARSLDWTKVTLDGRPLSTIQQYSKTFFVLPLRGKLSFWEAGTTKAGYPYNYNTTASDQLLVENAAGHRVAISTYTTSLGAGPVSISAVAVLAPHSVLALLEDTMDYPARAHTFDDFCPECRPLGLQGCAFQSTVAELQRLKMKVGKTREL

SEQ ID NO: 10 - protein, 115 aa, synthetic construct
DVQLQESGGGLVQPGGSLRLSCAASGFTLSRSTMTWGRQAPGKGLEWVSDIYSSGSTTYADSVKGRFTISRDNAKNTVYLQMNSLKPEDTAVYYCAVVLPGREYRGQGTQVTVSS

SEQ ID NO: 11 - protein, 126 aa, synthetic construct
DVQLQESGGGLVQPGGSLRLSCAASGFSLDYYAIGWFRQAPGKEREGVSCVSGREGSTIYTNSVKGRFTISRDNAKNTVHLQMNSLKPEDTAVYYCAAAGWNGLGCPPSLYEYDYWGQGTQVTVSS

SEQ ID NO: 12 - protein, 126 aa, synthetic construct
DVQLQESGGGLVQPGGSLRLSCAASTFTLDYYAIGWFRQAPGKEREGVSCISSRGGSTDYADSVKGRFTISRDNAKNTVYLQMSSLQPEDTAVYYCAAAGWAGYGCPPNRYEYDYWGQGTQVTVSS

SEQ ID NO: 13 - protein, 131 aa, synthetic construct
DVQLQESGGGLVQPGGSLRLSCAASGFTLDYYTIGWFRQAPGKEREGVSCISSSDDSTYYADSVKGRFTISRDNAKNTVFLQMNSLKPEDTAVYSCAAVPRHTGISPVLAMCASSVWYDYWGQGTQVTVSS

SEQ ID NO: 14 - protein, 126 aa, synthetic construct
DVQLQESGGGLVQPGGSLRLSCAASGFTLDYYAVGWFRQAPGKEREGVSCLSGRNGSPYYANSGKGRFTISRDNAENTVYLQMTGLEPEDTAVYYCAAAGWNGLGCPPSLYEYDYWGQGTQVTVSS

SEQ ID NO: 15 - protein, 125 aa, synthetic construct
DVQLQESGGGLVQPGGSLRLSCAASGFTLDYYAIGWFRQAPGKEREGVSCISGRSDSTNYADSVKGRFTISRDNAKNAVYLQMNSLKPEDTAVYYCAVSGWAGNGCPPIYEYDYWGQGTQVTVSS

SEQ ID NO: 16 - protein, 126 aa, synthetic construct
DVQLQESGGGLVQPGGSLRLSCAASGFTLDYYAIGWFRQAPGKEREEVSCISSRGGSTNYPDSVKGRFTISRDNAKNTVYLQMNSLRPEDTAVYYCAAAGWAGFGCPPNRYEYDYWGQGTQVTVSS

SEQ ID NO: 17 - protein, 126 aa, synthetic construct
DVQLQESGGGLVQPGGSLRLSCAGSGFTLDYYAIGWFRQAPGKEREGVSCISGRGGSTNYADSTKGRFTISRDNAKNTVYLQMNSLKPEDTAVYYCAAAGWAGNVCPPNRYEYDYWGQGTQVTVSS

SEQ ID NO: 18 - protein, 126 aa, synthetic construct
DVQLQESGGGLVQPGGSLRLSCAASGFTLDYYAIGWFRQAPGEVREEVSCISGRGDSTNYAHSMKGRFTISRDNAKNTVYLQINSLKPEDTAVYYCAAAGWAGYECPANRYEYDYWGQGTQVTVSS

SEQ ID NO: 19 - protein, 126 aa, synthetic construct
DVQLQESGGGLVQPGGSLRLSCAASGFTLDYYAIGWFRQAPGKEREEVSCISGRGSSTNYADSVKGRFTVSRDNAKNTVYLQINSLKPEDTAVYYCAAAGWAGYGCPANRYEYDYWGQGTQVTVSS

SEQ ID NO: 20 - protein, 126 aa, synthetic construct
DVQLQESGGGLVQPGGSTRLSCAASGFTLDYYAIGWFRQAPGKEREEVSCMSSRGGSTNYVDSVQGRFTLSRDNAKNTVYLQMNSLKPEDTAVYYCAAAGWAGNGCPPNRYEYDYWGQGTQVTVSS

SEQ ID NO: 21 - protein, 126 aa, synthetic construct
DVQLQESGGGLVQPGGSLRLSCAASGFTLDYYAIGWFRQAPGKEREGVSCISSRGGSTNTPDSVKGRFTISRDNAKNTVYLQMNSLRPEDTAVYYCAAAGWAGFGCPPNRYEYDYWGQGTQVTVSS

SEQ ID NO: 22 - protein, 115 aa, synthetic construct
DVQLQESGGGLVQPGGSLRLSCAASGFTLSRSTMTWGRQAPGKGLEWVSDIYRSGSTTYADSVKGRFTISRDDAKNTVYLQMNSLKPEDTAVYYCAVVLPGREYRGQGTQVTVSS

SEQ ID NO: 23 - protein, 126 aa, synthetic construct
DVQLQESGGGLVQPGGSLRLSCAASTFTLDYYAIGWFRQAPGKEREEVSCISSRSGSTNYPDSVKGRFTISRDNAKNTVYLQMNSLKPEDTAVYYCAAAGWAGYGCPANRYEYDYWGQGTQVTVSS

SEQ ID NO: 24 - protein, 126 aa, synthetic construct
DVQLQESGGGLVQPGGSLRLSCAASGFTLDHYAIGWFRQAPGKEREGISCISSRRGSTNYEDSVKGRFTISRDNAKNTVYLQMNSLKPEDTAVYYCAAAGWAGYMCPPNRYEYDYWGQGTQVTVSS

SEQ ID NO: 25 - protein, 126 aa, synthetic construct
DVQLQESGGGLVQPGGSLRLSCAASRFTLDYYAIGWFRQAPGKEREEVSCISSRAGSTNYQDSVKGRFTISRDNAKNTVYLQMNSLKPEDTAVYYCAAAGWAGNACPPNRYEYDYWGQGTQVTVSS

SEQ ID NO: 26 - protein, 126 aa, synthetic construct
DVQLQESGGGLVQPGGSLRLSCAASGFTLDYYAIGWFRQAPGKEREGVSCISGRRGSTIYANSVKGRFTNSRDNAKNTVYLQINSLKPEDTAVYYCAAAGWNGLGCPPSLDEYDYWGQGTQVTVSS

SEQ ID NO: 27 - protein, 126 aa, synthetic construct
DVQLQESGGGLVQPGGSLRLSCAASGFTLDYYAIGWFRQAPGKEREGVSCVSGRHGSTIYANSVKGRFTNSRDNAKNTVYLQINSLKPEDTAVYYCAAAGWNGLGCPPSLDEYDYWGQGTQVTVSS

SEQ ID NO: 28 - protein, 126 aa, synthetic construct
DVQLQESGGGLVQPGGSLRLSCAASGLTLDYYNIGWFRQAPGKEREGVSCISVSGGVTNYADSVMGRFTVSRDNAKNTVYLQMNSLKPEDTAVYYCAAVSLPFVPMLGCPEGYDYWGQGTQVTVSS

SEQ ID NO: 29 - protein, 124 aa, synthetic construct
DVQLQESGGGLVQPGGSLRLSCAASGFTLDEYTIGWFRQAPGKERQGVSCISSRGGRTNYADSVKGRFTISRDNAKNTVYLLMNSLEPEDTAVYYCAAASYYDDCRVPAWYDYWGQGTQVTVSS

SEQ ID NO: 30 - protein, 623 aa, synthetic construct
MGTVNKPVVGVLMGFGIITGTLRITNPVRASVLRYDDFHIDEDKLDTNSVYEPYYHSDHAESSWVNRGESSRKAYDHNSPYIWPRNDYDGFLENAHEHHGVYNQGRGIDSGERLMQPTQMSAQEDLGDDTGIHVIPTLNGDDRHKIVNVDQRQYGDVFKGDLNPKPQGQRLIEVSVEENHPFTLRAPIQRIYGVRYTETWSFLPSLTCTGDAAPAIQHICLKHTTCFQDVVVDVDCAENTKEDQLAEISYRFQGKKEADQPWIVVNTSTLFDELELDPPEIEPGVLKVLRTEKQYLGVYIWNMRGSDGTSTYATFLVTWKGDEKTRNPTPAVTPQPRGAEFHMWNYHSHVFSVGDTFSLAMHLQYKIHEAPFDLLLEWLYVPIDPTCQPMRLYSTCLYHPNAPQCLSHMNSGCTFTSPHLAQRVASTVYQNCEHADNYTAYCLGISHMEPSFGLILHDGGTTLKFVDTPESLSGLYVFVVYFNGHVEAVAYTVVSTVDHFVNAIEERGFPPTAGQPPATTKPKEITPVNPGTSPLIRYAAWTGGLAAVVLLCLVIFLICTAKRMRVKAYRVDKSPYNQSMYYAGLPVDDFEDSESTDTEEEFGNAIGGSHGGSSYTVYIDKTR

SEQ ID NO: 31 - protein, 20 aa, synthetic construct
KFLVNVALVFMVVYISYIYA

SEQ ID NO: 32 - protein, 375 aa, synthetic construct
KFLVNVALVFMVVYISYIYADVQLQESGGGLVQPGGSLRLSCAASTFTLDYYAIGWFRQAPGKEREGVSCISSRGGSTDYADSVKGRFTISRDNAKNTVYLQMSSLQPEDTAVYYCAAAGWAGYGCPPNRYEYDYWGQGTQVTVSSRVQPTESIVRFPNITNLCPFGEVFNATRFASVYAWNRKRISNCVADYSVLYNSASFSTFKCYGVSPTKLNDLCFTNVYADSFVIRGDEVRQIAPGQTGTIADYNYKLPDDFTGCVIAWNSNNLDSKVGGNYNYLYRLFRKSNLKPFERDISTEIYQAGSTPCNGVKGFNCYFPLQSYGFQPTYGVGYQPYRVVVLSFELLHAPATVCGPKKSTNLVKNKCVNFHHHHHH

SEQ ID NO: 33 - protein, 671 aa, synthetic construct
KFLVNVALVFMVVYISYIYADVQLQESGGGLVQPGGSLRLSCAASGFTLDYYAIGWFRQAPGKEREGVSCISGRRGSTIYANSVKGRFTNSRDNAKNTVYLQINSLKPEDTAVYYCAAAGWNGLGCPPSLDEYDYWGQGTQVTVSSRITNPVRASVLRYDDFHIDEDKLDTNSVYEPYYHSDHAESSWVNRGESSRKAYDHNSPYIWPRNDYDGFLENAHEHHGVYNQGRGIDSGERLMQPTQMSAQEDLGDDTGIHVIPTLNGDDRHKIVNVDQRQYGDVFKGDLNPKPQGQRLIEVSVEENHPFTLRAPIQRIYGVRYTETWSFLPSLTCTGDAAPAIQHICLKHTTCFQDVVVDVDCAENTKEDQLAEISYRFQGKKEADQPWIVVNTSTLFDELELDPPEIEPGVLKVLRTEKQYLGVYIWNMRGSDGTSTYATFLVTWKGDEKTRNPTPAVTPQPRGAEFHMWNYHSHVFSVGDTFSLAMHLQYKIHEAPFDLLLEWLYVPIDPTCQPMRLYSTCLYHPNAPQCLSHMNSGCTFTSPHLAQRVASTVYQNCEHADNYTAYCLGISHMEPSFGLILHDGGTTLKFVDTPESLSGLYVFVVYFNGHVEAVAYTVVSTVDHFVNAIEERGFPPTAGQPPATTKPKEITPVNPGTSPLLRHHHHHHHHHH

SEQ ID NO: 34 - protein, 624 aa, synthetic construct
AENLAVGIGAVFLGFLGAAGSTMGAASMTLTVQARNLLSGIVQQQSNLLRAPEAQQHLLKLTVWGIKQLQARVLAVERYLRDQQLLGIWGCSGKLICTTNVPNLWVTVYYGVPVWKDAETTLFCASDAKAYETEKHNVWATHACVPTDPNPQEIHLENVTEEFNMWKNNMVEQMHTDIISLWDQSLKPCVKLTPLCVTLQCTNVTNNITDDMRGELKNCSFNMTTELRDKKQKVYSLFYRLDVVQINENQGNRSNNSNKEYRLINCNTSAITQACPKVSFEPIPIHYCAPAGFAILKCKDKKFNGTGPCPSVSTVQCTHGIKPVVSTQLLLNGSLAEEEVMIRSENITNNAKNILVQFNTPVQINCTRPNNNTRKSIRIGPGQAFYATGDIIGDIRQAHCNVSKATWNETLGKVVKQLRKHFGNNTIIRFANSSGGDLEVTTHSFNCGGEFFYCNTSGLFNSTWISNTSVQGSNSTGSNDSITLPCRIKQIINMWQRIGQAMYAPPIQGVIRCVSNITGLILTRDGGSTNSTTETFRPGGGDMRDNWRSELYKYKVVKIEPLGVAPTRRNLSEIWDNMTWLQWDKEISNYTQIIYGLLEESQNQQEKNEQDLLALDHHHHHHHH

SEQ ID NO: 35 - protein, 640 aa, synthetic construct
AENLWVTVYYGVPVWKDAETTLFCASDAKAYETEKHNVWATHACVPTDPNPQEIHLENVTEEFNMWKNNMVEQMHTDIISLWDQSLKPCVKLTPLCVTLQCTNVTNNITDDMRGELKNCSFNMTTELRDKKQKVYSLFYRLDVVQINENQGNRSNNSNKEYRLINCNTSAITQACPKVSFEPIPIHYCAPAGFAILKCKDKKFNGTGPCPSVSTVQCTHGIKPVVSTQLLLNGSLAEEEVMIRSENITNNAKNILVQFNTPVQINCTRPNNNTRKSIRIGPGQAFYATGDIIGDIRQAHCNVSKATWNETLGKVVKQLRKHFGNNTIIRFANSSGGDLEVTTHSFNCGGEFFYCNTSGLFNSTWISNTSVQGSNSTGSNDSITLPCRIKQIINMWQRIGQAMYAPPIQGVIRCVSNITGLILTRDGGSTNSTTETFRPGGGDMRDNWRSELYKYKVVKIEPLGVAPTRCKRRVVGRRRRRRAVGIGAVFLGFLGAAGSTMGAASMTLTVQARNLLSGIVQQQSNLLRAPEAQQHLLKLTVWGIKQLQARVLAVERYLRDQQLLGIWGCSGKLICCTNVPWNSSWSNRNLSEIWDNMTWLQWDKEISNYTQIIYGLLEESQNQQEKNEQDLLALDHHHHHH

SEQ ID NO: 36 - protein, 765 aa, synthetic construct
DVQLQESGGGLVQPGGSLRLSCAASGFTLDYYAIGWFRQAPGKEREGVSCISSRGGSTNTPDSVKGRFTISRDNAKNTVYLQMNSLRPEDTAVYYCAAAGWAGFGCPPNRYEYDYWGQGTQVTVSSGGGGSGGGGSGGGGSAENLAVGIGAVFLGFLGAAGSTMGAASMTLTVQARNLLSGIVQQQSNLLRAPEAQQHLLKLTVWGIKQLQARVLAVERYLRDQQLLGIWGCSGKLICTTNVPNLWVTVYYGVPVWKDAETTLFCASDAKAYETEKHNVWATHACVPTDPNPQEIHLENVTEEFNMWKNNMVEQMHTDIISLWDQSLKPCVKLTPLCVTLQCTNVTNNITDDMRGELKNCSFNMTTELRDKKQKVYSLFYRLDVVQINENQGNRSNNSNKEYRLINCNTSAITQACPKVSFEPIPIHYCAPAGFAILKCKDKKFNGTGPCPSVSTVQCTHGIKPVVSTQLLLNGSLAEEEVMIRSENITNNAKNILVQFNTPVQINCTRPNNNTRKSIRIGPGQAFYATGDIIGDIRQAHCNVSKATWNETLGKVVKQLRKHFGNNTIIRFANSSGGDLEVTTHSFNCGGEFFYCNTSGLFNSTWISNTSVQGSNSTGSNDSITLPCRIKQIINMWQRIGQAMYAPPIQGVIRCVSNITGLILTRDGGSTNSTTETFRPGGGDMRDNWRSELYKYKVVKIEPLGVAPTRRNLSEIWDNMTWLQWDKEISNYTQIIYGLLEESQNQQEKNEQDLLALDHHHHHHHH

SEQ ID NO: 37 - protein, 35 aa, synthetic construct
MDAMKRGLCCVLLLCGAVFVSPSQEIHARFRRGAR

SEQ ID NO: 38 - protein, 19 aa, synthetic construct
MGWSCIILFLVATATGVHS

SEQ ID NO: 39 - protein, 15 aa, synthetic construct
GGGGSGGGGSGGGGS

SEQ ID NO: 40 - protein, 239 aa, synthetic construct
IALTLFNLADTLLGGLPTELISSAGGQLFYSRPVVSANGEPTVKLYTSVENAQQDKGIAIPHDIDLGESRVVIQDYDNQHEQDRPTPSPAPSRPFSVLRANDVLWLSLTAAEYDQSTYGSSTGPVYVSDSVTLVNVATGAQAVARSLDWTKVTLDGRPLSTIQQYSKTFFVLPLRGKLSFWEAGTTKAGYPYNYNTTASDQLLVENAAGHRVAISTYTTSLGAGPVSISAVAVLAPHSV

SEQ ID NO: 41 - protein, 495 aa, synthetic construct
AVAPAHDTPPVPDVDSRGAILRRQYNLSTSPLTSSVATGTNLVLYAAPLSPLLPLQDGTNTHIMATEASNYAQYRVARATIRYRPLVPNAVGGYAISISFWPQTTTTPTSVDMNSITSTDVRILVQPGIASELVIPSERLHYRNQGWRSVETSGVAEEEATSGLVMLCIHGSPVNSYTNTPYTGALGLLDFALELEFRNLTPGNTNTRVSRYSSTARHRLRRGADGTAELTTTAATRFMKDLYFTSTNGVGEIGRGIALTLFNLADTLLGGLPTELISSAGGQLFYSRPVVSANGEPTVKLYTSVENAQQDKGIAIPHDIDLGESRVVIQDYDNQHEQDRPTPSPAPSRPFSVLRANDVLWLSLTAAEYDQSTYGSSTGPVYVSDSVTLVNVATGAQAVARSLDWTKVTLDGRPLSTIQQYSKTFFVLPLRGKLSFWEAGTTKAGYPYNYNTTASDQLLVENAAGHRVAISTYTTSLGAGPVSISAVAVLAPHSV

SEQ ID NO: 42 - protein, 355 aa, synthetic construct
DVQLQESGGGLVQPGGSLRLSCAASTFTLDYYAIGWFRQAPGKEREGVSCISSRGGSTDYADSVKGRFTISRDNAKNTVYLQMSSLQPEDTAVYYCAAAGWAGYGCPPNRYEYDYWGQGTQVTVSSRVQPTESIVRFPNITNLCPFGEVFNATRFASVYAWNRKRISNCVADYSVLYNSASFSTFKCYGVSPTKLNDLCFTNVYADSFVIRGDEVRQIAPGQTGKIADYNYKLPDDFTGCVIAWNSNNLDSKVGGNYNYLYRLFRKSNLKPFERDISTEIYQAGSTPCNGVEGFNCYFPLQSYGFQPTNGVGYQPYRVVVLSFELLHAPATVCGPKKSTNLVKNKCVNFHHHHHH

SEQ ID NO: 43 - protein, 354 aa, synthetic construct
DVQLQESGGGLVQPGGSLRLSCAASGFTLDYYAIGWFRQAPGKEREGVSCISGRSDSTNYADSVKGRFTISRDNAKNAVYLQMNSLKPEDTAVYYCAVSGWAGNGCPPIYEYDYWGQGTQVTVSSRVQPTESIVRFPNITNLCPFGEVFNATRFASVYAWNRKRISNCVADYSVLYNSASFSTFKCYGVSPTKLNDLCFTNVYADSFVIRGDEVRQIAPGQTGKIADYNYKLPDDFTGCVIAWNSNNLDSKVGGNYNYLYRLFRKSNLKPFERDISTEIYQAGSTPCNGVEGFNCYFPLQSYGFQPTNGVGYQPYRVVVLSFELLHAPATVCGPKKSTNLVKNKCVNFHHHHHH

SEQ ID NO: 44 - protein, 344 aa, synthetic construct
DVQLQESGGGLVQPGGSLRLSCAASGFTLSRSTMTWGRQAPGKGLEWVSDIYSSGSTTYADSVKGRFTISRDNAKNTVYLQMNSLKPEDTAVYYCAVVLPGREYRGQGTQVTVSSRVQPTESIVRFPNITNLCPFGEVFNATRFASVYAWNRKRISNCVADYSVLYNSASFSTFKCYGVSPTKLNDLCFTNVYADSFVIRGDEVRQIAPGQTGKIADYNYKLPDDFTGCVIAWNSNNLDSKVGGNYNYLYRLFRKSNLKPFERDISTEIYQAGSTPCNGVEGFNCYFPLQSYGFQPTNGVGYQPYRVVVLSFELLHAPATVCGPKKSTNLVKNKCVNFHHHHHH

SEQ ID NO: 45 - protein, 355 aa, synthetic construct
DVQLQESGGGLVQPGGSLRLSCAASGFSLDYYAIGWFRQAPGKEREGVSCVSGREGSTIYTNSVKGRFTISRDNAKNTVHLQMNSLKPEDTAVYYCAAAGWNGLGCPPSLYEYDYWGQGTQVTVSSRVQPTESIVRFPNITNLCPFGEVFNATRFASVYAWNRKRISNCVADYSVLYNSASFSTFKCYGVSPTKLNDLCFTNVYADSFVIRGDEVRQIAPGQTGKIADYNYKLPDDFTGCVIAWNSNNLDSKVGGNYNYLYRLFRKSNLKPFERDISTEIYQAGSTPCNGVEGFNCYFPLQSYGFQPTNGVGYQPYRVVVLSFELLHAPATVCGPKKSTNLVKNKCVNFHHHHHH

SEQ ID NO: 46 - protein, 355 aa, synthetic construct
DVQLQESGGGLVQPGGSLRLSCAASGFTLDYYAIGWFRQAPGKEREEVSCISGRGSSTNYADSVKGRFTVSRDNAKNTVYLQINSLKPEDTAVYYCAAAGWAGYGCPANRYEYDYWGQGTQVTVSSRVQPTESIVRFPNITNLCPFGEVFNATRFASVYAWNRKRISNCVADYSVLYNSASFSTFKCYGVSPTKLNDLCFTNVYADSFVIRGDEVRQIAPGQTGKIADYNYKLPDDFTGCVIAWNSNNLDSKVGGNYNYLYRLFRKSNLKPFERDISTEIYQAGSTPCNGVEGFNCYFPLQSYGFQPTNGVGYQPYRVVVLSFELLHAPATVCGPKKSTNLVKNKCVNFHHHHHH

SEQ ID NO: 47 - protein, 355 aa, synthetic construct
DVQLQESGGGLVQPGGSLRLSCAASGFTLDYYAIGWFRQAPGEVREEVSCISGRGDSTNYAHSMKGRFTISRDNAKNTVYLQINSLKPEDTAVYYCAAAGWAGYECPANRYEYDYWGQGTQVTVSSRVQPTESIVRFPNITNLCPFGEVFNATRFASVYAWNRKRISNCVADYSVLYNSASFSTFKCYGVSPTKLNDLCFTNVYADSFVIRGDEVRQIAPGQTGKIADYNYKLPDDFTGCVIAWNSNNLDSKVGGNYNYLYRLFRKSNLKPFERDISTEIYQAGSTPCNGVEGFNCYFPLQSYGFQPTNGVGYQPYRVVVLSFELLHAPATVCGPKKSTNLVKNKCVNFHHHHHH

SEQ ID NO: 48 - protein, 355 aa, synthetic construct
DVQLQESGGGLVQPGGSLRLSCAGSGFTLDYYAIGWFRQAPGKEREGVSCISGRGGSTNYADSTKGRFTISRDNAKNTVYLQMNSLKPEDTAVYYCAAAGWAGNVCPPNRYEYDYWGQGTQVTVSSRVQPTESIVRFPNITNLCPFGEVFNATRFASVYAWNRKRISNCVADYSVLYNSASFSTFKCYGVSPTKLNDLCFTNVYADSFVIRGDEVRQIAPGQTGKIADYNYKLPDDFTGCVIAWNSNNLDSKVGGNYNYLYRLFRKSNLKPFERDISTEIYQAGSTPCNGVEGFNCYFPLQSYGFQPTNGVGYQPYRVVVLSFELLHAPATVCGPKKSTNLVKNKCVNFHHHHHH

SEQ ID NO: 49 - protein, 355 aa, synthetic construct
DVQLQESGGGLVQPGGSLRLSCAASGFTLDYYAIGWFRQAPGKEREEVSCISSRGGSTNYPDSVKGRFTISRDNAKNTVYLQMNSLRPEDTAVYYCAAAGWAGFGCPPNRYEYDYWGQGTQVTVSSRVQPTESIVRFPNITNLCPFGEVFNATRFASVYAWNRKRISNCVADYSVLYNSASFSTFKCYGVSPTKLNDLCFTNVYADSFVIRGDEVRQIAPGQTGKIADYNYKLPDDFTGCVIAWNSNNLDSKVGGNYNYLYRLFRKSNLKPFERDISTEIYQAGSTPCNGVEGFNCYFPLQSYGFQPTNGVGYQPYRVVVLSFELLHAPATVCGPKKSTNLVKNKCVNFHHHHHH

SEQ ID NO: 50 - protein, 755 aa, synthetic construct
DVQLQESGGGLVQPGGSLRLSCAASGFTLDYYAIGWFRQAPGKEREGVSCVSGRHGSTIYANSVKGRFTNSRDNAKNTVYLQINSLKPEDTAVYYCAAAGWNGLGCPPSLDEYDYWGQGTQVTVSSMGTVNKPVVGVLMGFGIITGTLRITNPVRASVLRYDDFHIDEDKLDTNSVYEPYYHSDHAESSWVNRGESSRKAYDHNSPYIWPRNDYDGFLENAHEHHGVYNQGRGIDSGERLMQPTQMSAQEDLGDDTGIHVIPTLNGDDRHKIVNVDQRQYGDVFKGDLNPKPQGQRLIEVSVEENHPFTLRAPIQRIYGVRYTETWSFLPSLTCTGDAAPAIQHICLKHTTCFQDVVVDVDCAENTKEDQLAEISYRFQGKKEADQPWIVVNTSTLFDELELDPPEIEPGVLKVLRTEKQYLGVYIWNMRGSDGTSTYATFLVTWKGDEKTRNPTPAVTPQPRGAEFHMWNYHSHVFSVGDTFSLAMHLQYKIHEAPFDLLLEWLYVPIDPTCQPMRLYSTCLYHPNAPQCLSHMNSGCTFTSPHLAQRVASTVYQNCEHADNYTAYCLGISHMEPSFGLILHDGGTTLKFVDTPESLSGLYVFVVYFNGHVEAVAYTVVSTVDHFVNAIEERGFPPTAGQPPATTKPKEITPVNPGTSPLIRYAAWTGGLAAVVLLCLVIFLICTAKRMRVKAYRVDKSPYNQSMYYAGLPVDDFEDSESTDTEEEFGNAIGGSHGGSSYTVYIDKTRHHHHHH

SEQ ID NO: 51 - protein, 755 aa, synthetic construct
DVQLQESGGGLVQPGGSLRLSCAASTFTLDYYAIGWFRQAPGKEREEVSCISSRSGSTNYPDSVKGRFTISRDNAKNTVYLQMNSLKPEDTAVYYCAAAGWAGYGCPANRYEYDYWGQGTQVTVSSMGTVNKPVVGVLMGFGIITGTLRITNPVRASVLRYDDFHIDEDKLDTNSVYEPYYHSDHAESSWVNRGESSRKAYDHNSPYIWPRNDYDGFLENAHEHHGVYNQGRGIDSGERLMQPTQMSAQEDLGDDTGIHVIPTLNGDDRHKIVNVDQRQYGDVFKGDLNPKPQGQRLIEVSVEENHPFTLRAPIQRIYGVRYTETWSFLPSLTCTGDAAPAIQHICLKHTTCFQDVVVDVDCAENTKEDQLAEISYRFQGKKEADQPWIVVNTSTLFDELELDPPEIEPGVLKVLRTEKQYLGVYIWNMRGSDGTSTYATFLVTWKGDEKTRNPTPAVTPQPRGAEFHMWNYHSHVFSVGDTFSLAMHLQYKIHEAPFDLLLEWLYVPIDPTCQPMRLYSTCLYHPNAPQCLSHMNSGCTFTSPHLAQRVASTVYQNCEHADNYTAYCLGISHMEPSFGLILHDGGTTLKFVDTPESLSGLYVFVVYFNGHVEAVAYTVVSTVDHFVNAIEERGFPPTAGQPPATTKPKEITPVNPGTSPLIRYAAWTGGLAAVVLLCLVIFLICTAKRMRVKAYRVDKSPYNQSMYYAGLPVDDFEDSESTDTEEEFGNAIGGSHGGSSYTVYIDKTRHHHHHH

SEQ ID NO: 52 - protein, 755 aa, synthetic construct
DVQLQESGGGLVQPGGSLRLSCAASGFTLDYYAIGWFRQAPGKEREGVSCISSRGGSTNTPDSVKGRFTISRDNAKNTVYLQMNSLRPEDTAVYYCAAAGWAGFGCPPNRYEYDYWGQGTQVTVSSMGTVNKPVVGVLMGFGIITGTLRITNPVRASVLRYDDFHIDEDKLDTNSVYEPYYHSDHAESSWVNRGESSRKAYDHNSPYIWPRNDYDGFLENAHEHHGVYNQGRGIDSGERLMQPTQMSAQEDLGDDTGIHVIPTLNGDDRHKIVNVDQRQYGDVFKGDLNPKPQGQRLIEVSVEENHPFTLRAPIQRIYGVRYTETWSFLPSLTCTGDAAPAIQHICLKHTTCFQDVVVDVDCAENTKEDQLAEISYRFQGKKEADQPWIVVNTSTLFDELELDPPEIEPGVLKVLRTEKQYLGVYIWNMRGSDGTSTYATFLVTWKGDEKTRNPTPAVTPQPRGAEFHMWNYHSHVFSVGDTFSLAMHLQYKIHEAPFDLLLEWLYVPIDPTCQPMRLYSTCLYHPNAPQCLSHMNSGCTFTSPHLAQRVASTVYQNCEHADNYTAYCLGISHMEPSFGLILHDGGTTLKFVDTPESLSGLYVFVVYFNGHVEAVAYTVVSTVDHFVNAIEERGFPPTAGQPPATTKPKEITPVNPGTSPLIRYAAWTGGLAAVVLLCLVIFLICTAKRMRVKAYRVDKSPYNQSMYYAGLPVDDFEDSESTDTEEEFGNAIGGSHGGSSYTVYIDKTRHHHHHH

SEQ ID NO: 53 - protein, 755 aa, synthetic construct
DVQLQESGGGLVQPGGSLRLSCAASGFTLDYYAIGWFRQAPGKEREGVSCISGRRGSTIYANSVKGRFTNSRDNAKNTVYLQINSLKPEDTAVYYCAAAGWNGLGCPPSLDEYDYWGQGTQVTVSSMGTVNKPVVGVLMGFGIITGTLRITNPVRASVLRYDDFHIDEDKLDTNSVYEPYYHSDHAESSWVNRGESSRKAYDHNSPYIWPRNDYDGFLENAHEHHGVYNQGRGIDSGERLMQPTQMSAQEDLGDDTGIHVIPTLNGDDRHKIVNVDQRQYGDVFKGDLNPKPQGQRLIEVSVEENHPFTLRAPIQRIYGVRYTETWSFLPSLTCTGDAAPAIQHICLKHTTCFQDVVVDVDCAENTKEDQLAEISYRFQGKKEADQPWIVVNTSTLFDELELDPPEIEPGVLKVLRTEKQYLGVYIWNMRGSDGTSTYATFLVTWKGDEKTRNPTPAVTPQPRGAEFHMWNYHSHVFSVGDTFSLAMHLQYKIHEAPFDLLLEWLYVPIDPTCQPMRLYSTCLYHPNAPQCLSHMNSGCTFTSPHLAQRVASTVYQNCEHADNYTAYCLGISHMEPSFGLILHDGGTTLKFVDTPESLSGLYVFVVYFNGHVEAVAYTVVSTVDHFVNAIEERGFPPTAGQPPATTKPKEITPVNPGTSPLIRYAAWTGGLAAVVLLCLVIFLICTAKRMRVKAYRVDKSPYNQSMYYAGLPVDDFEDSESTDTEEEFGNAIGGSHGGSSYTVYIDKTRHHHHHH

SEQ ID NO: 54 - protein, 755 aa, synthetic construct
DVQLQESGGGLVQPGGSLRLSCAASGLTLDYYNIGWFRQAPGKEREGVSCISVSGGVTNYADSVMGRFTVSRDNAKNTVYLQMNSLKPEDTAVYYCAAVSLPFVPMLGCPEGYDYWGQGTQVTVSSMGTVNKPVVGVLMGFGIITGTLRITNPVRASVLRYDDFHIDEDKLDTNSVYEPYYHSDHAESSWVNRGESSRKAYDHNSPYIWPRNDYDGFLENAHEHHGVYNQGRGIDSGERLMQPTQMSAQEDLGDDTGIHVIPTLNGDDRHKIVNVDQRQYGDVFKGDLNPKPQGQRLIEVSVEENHPFTLRAPIQRIYGVRYTETWSFLPSLTCTGDAAPAIQHICLKHTTCFQDVVVDVDCAENTKEDQLAEISYRFQGKKEADQPWIVVNTSTLFDELELDPPEIEPGVLKVLRTEKQYLGVYIWNMRGSDGTSTYATFLVTWKGDEKTRNPTPAVTPQPRGAEFHMWNYHSHVFSVGDTFSLAMHLQYKIHEAPFDLLLEWLYVPIDPTCQPMRLYSTCLYHPNAPQCLSHMNSGCTFTSPHLAQRVASTVYQNCEHADNYTAYCLGISHMEPSFGLILHDGGTTLKFVDTPESLSGLYVFVVYFNGHVEAVAYTVVSTVDHFVNAIEERGFPPTAGQPPATTKPKEITPVNPGTSPLIRYAAWTGGLAAVVLLCLVIFLICTAKRMRVKAYRVDKSPYNQSMYYAGLPVDDFEDSESTDTEEEFGNAIGGSHGGSSYTVYIDKTRHHHHHH

SEQ ID NO: 55 - protein, 744 aa, synthetic construct
DVQLQESGGGLVQPGGSLRLSCAASGFTLSRSTMTWGRQAPGKGLEWVSDIYRSGSTTYADSVKGRFTISRDDAKNTVYLQMNSLKPEDTAVYYCAVVLPGREYRGQGTQVTVSSMGTVNKPVVGVLMGFGIITGTLRITNPVRASVLRYDDFHIDEDKLDTNSVYEPYYHSDHAESSWVNRGESSRKAYDHNSPYIWPRNDYDGFLENAHEHHGVYNQGRGIDSGERLMQPTQMSAQEDLGDDTGIHVIPTLNGDDRHKIVNVDQRQYGDVFKGDLNPKPQGQRLIEVSVEENHPFTLRAPIQRIYGVRYTETWSFLPSLTCTGDAAPAIQHICLKHTTCFQDVVVDVDCAENTKEDQLAEISYRFQGKKEADQPWIVVNTSTLFDELELDPPEIEPGVLKVLRTEKQYLGVYIWNMRGSDGTSTYATFLVTWKGDEKTRNPTPAVTPQPRGAEFHMWNYHSHVFSVGDTFSLAMHLQYKIHEAPFDLLLEWLYVPIDPTCQPMRLYSTCLYHPNAPQCLSHMNSGCTFTSPHLAQRVASTVYQNCEHADNYTAYCLGISHMEPSFGLILHDGGTTLKFVDTPESLSGLYVFVVYFNGHVEAVAYTVVSTVDHFVNAIEERGFPPTAGQPPATTKPKEITPVNPGTSPLIRYAAWTGGLAAVVLLCLVIFLICTAKRMRVKAYRVDKSPYNQSMYYAGLPVDDFEDSESTDTEEEFGNAIGGSHGGSSYTVYIDKTRHHHHHH

SEQ ID NO: 56 - protein, 755 aa, synthetic construct
DVQLQESGGGLVQPGGSLRLSCAASRFTLDYYAIGWFRQAPGKEREEVSCISSRAGSTNYQDSVKGRFTISRDNAKNTVYLQMNSLKPEDTAVYYCAAAGWAGNACPPNRYEYDYWGQGTQVTVSSMGTVNKPVVGVLMGFGIITGTLRITNPVRASVLRYDDFHIDEDKLDTNSVYEPYYHSDHAESSWVNRGESSRKAYDHNSPYIWPRNDYDGFLENAHEHHGVYNQGRGIDSGERLMQPTQMSAQEDLGDDTGIHVIPTLNGDDRHKIVNVDQRQYGDVFKGDLNPKPQGQRLIEVSVEENHPFTLRAPIQRIYGVRYTETWSFLPSLTCTGDAAPAIQHICLKHTTCFQDVVVDVDCAENTKEDQLAEISYRFQGKKEADQPWIVVNTSTLFDELELDPPEIEPGVLKVLRTEKQYLGVYIWNMRGSDGTSTYATFLVTWKGDEKTRNPTPAVTPQPRGAEFHMWNYHSHVFSVGDTFSLAMHLQYKIHEAPFDLLLEWLYVPIDPTCQPMRLYSTCLYHPNAPQCLSHMNSGCTFTSPHLAQRVASTVYQNCEHADNYTAYCLGISHMEPSFGLILHDGGTTLKFVDTPESLSGLYVFVVYFNGHVEAVAYTVVSTVDHFVNAIEERGFPPTAGQPPATTKPKEITPVNPGTSPLIRYAAWTGGLAAVVLLCLVIFLICTAKRMRVKAYRVDKSPYNQSMYYAGLPVDDFEDSESTDTEEEFGNAIGGSHGGSSYTVYIDKTRHHHHHH

SEQ ID NO: 57 - protein, 8 aa, synthetic construct
TFTLDYYA

SEQ ID NO: 58 - protein, 8 aa, synthetic construct
ISSRGGST

SEQ ID NO: 59 - protein, 19 aa, synthetic construct
AAAGWAGYGCPPNRYEYDY

SEQ ID NO: 60 - protein, 8 aa, synthetic construct
GFTLDYYA

SEQ ID NO: 61 - protein, 8 aa, synthetic construct
ISSRGGST

SEQ ID NO: 62 - protein, 19 aa, synthetic construct
AAAGWAGFGCPPNRYEYDY

SEQ ID NO: 63 - protein, 374 aa, synthetic construct
MGWSCIILFLVATATGVHSEVQLVESGGGLVQPGGSLRLSCSASTFTLDYYAIGWVRQAPGKGLEYVSCISSRGGSTDYADSVKGRFTISRDNSKNTLYLQMSSLRAEDTAVYYCAAAGWAGYGCPPNRYEYDYWGQGTLVTVSSRVQPTESIVRFPNITNLCPFGEVFNATRFASVYAWNRKRISNCVADYSVLYNSASFSTFKCYGVSPTKLNDLCFTNVYADSFVIRGDEVRQIAPGQTGTIADYNYKLPDDFTGCVIAWNSNNLDSKVGGNYNYLYRLFRKSNLKPFERDISTEIYQAGSTPCNGVKGFNCYFPLQSYGFQPTYGVGYQPYRVVVLSFELLHAPATVCGPKKSTNLVKNKCVNFHHHHHH

SEQ ID NO: 64 - protein, 374 aa, synthetic construct
MGWSCIILFLVATATGVHSEVQLLESGGGLVQPGGSLRLSCAASTFTLDYYAIGWVRQAPGKGLEWVSCISSRGGSTDYADSVKGRFTISRDNSKNTLYLQMNSLRAEDTAVYYCAAAGWAGYGCPPNRYEYDYWGQGTLVTVSSRVQPTESIVRFPNITNLCPFGEVFNATRFASVYAWNRKRISNCVADYSVLYNSASFSTFKCYGVSPTKLNDLCFTNVYADSFVIRGDEVRQIAPGQTGTIADYNYKLPDDFTGCVIAWNSNNLDSKVGGNYNYLYRLFRKSNLKPFERDISTEIYQAGSTPCNGVKGFNCYFPLQSYGFQPTYGVGYQPYRVVVLSFELLHAPATVCGPKKSTNLVKNKCVNFHHHHHH

SEQ ID NO: 65 - protein, 10 aa, synthetic construct
TFTLDYYAIG

SEQ ID NO: 66 - protein, 10 aa, synthetic construct
CISSRGGSTD

SEQ ID NO: 67 - protein, 17 aa, synthetic construct
AAAGWAGYGCPPNRYEY

SEQ ID NO: 68 - protein, 126 aa, synthetic construct
EVQLVESGGGLVQPGGSLRLSCSASTFTLDYYAIGWVRQAPGKGLEYVSCISSRGGSTDYADSVKGRFTISRDNSKNTLYLQMSSLRAEDTAVYYCAAAGWAGYGCPPNRYEYDYWGQGTLVTVSS

SEQ ID NO: 69 - protein, 126 aa, synthetic construct
EVQLLESGGGLVQPGGSLRLSCAASTFTLDYYAIGWVRQAPGKGLEWVSCISSRGGSTDYADSVKGRFTISRDNSKNTLYLQMNSLRAEDTAVYYCAAAGWAGYGCPPNRYEYDYWGQGTLVTVSS

SEQ ID NO: 70 - protein, 226 aa, synthetic construct
MENTTSGFLGPLLGLQAGFFLLTRILTIPQSLDLWWTSLNFLGGAPKCPGLNSQSPTSNHSPTSCPPICPGYRSMCLRRFIIFLFILLLCLIFLLVLLDYQGMLPVCPLLPGTPTTSTGPCKTCTSPAQGNSTFPSCCCTKPSDGNCICIPIPSSWAFARFLWEWASVRFSWLSLLVPFVQWFVGLSPIVWLSVIWMMWYWGRSLYNILSPFLPLLPIFFCLWVYI

SEQ ID NO: 71 - protein, 498 aa, synthetic construct
MSVWRPSEATVYLPPVPVSKVVSTDEYVSRTSIYYYAGSSRLLAVGNPYFSIKSPNNNKKVLVPKVSGLQYRVFRVRLPDPNKFGFPDTSFYNPDTQRLVWACVGLEIGRGQPLGVGVSGHPYLNKFDDTETSNRYPAQPGSDNRECLSMDYKQTQLCLIGCKPPTGEHWGKGVACNNNAAATDCPPLELFNSIIEDGDMVDTGFGCMDFGTLQANKSDVPIDICNSTCKYPDYLKMASEPYGDSLFFFLRREQMFVRHFFNRAGKLGEAVPDDLYIKGSGNTAVIQSSAFFPTPSGSIVTSESQLFNKPYWLQRAQGHNNGICWGNQLFVTVVDTTRSTNMTLCTEVTKEGTYKNDNFKEYVRHVEEYDLQFVFQLCKITLTAEIMTYIHTMDSNILEDWQFGLTPPPSASLQDTYRFVTSQAITCQKTAPPKEKEDPLNKYTFWEVNLKEKFSADLDQFPLGRKFLLQSGLKAKPRLKRSAPTTRAPSTKRKKVKK

SEQ ID NO: 72 - protein, 361 aa, synthetic construct
DVQLQESGGGLVQPGGSLRLSCAASGFTLSRSTMTWGRQAPGKGLEWVSDIYSSGSTTYADSVKGRFTISRDNAKNTVYLQMNSLKPEDTAVYYCAVVLPGREYRGQGTQVTVSSGGGGSGGGGSGGGGSRVQPTESIVRFPNITNLCPFGEVFNATRFASVYAWNRKRISNCVADYSVLYNSASFSTFKCYGVSPTKLNDLCFTNVYADSFVIRGDEVRQIAPGQTGKIADYNYKLPDDFTGCVIAWNSNNLDSKVGGNYNYLYRLFRKSNLKPFERDISTEIYQAGSTPCNGVEGFNCYFPLQSYGFQPTNGVGYQPYRVVVLSFELLHAPATVCGPKKSTNLVKNKCVNFHHHHHHHH

SEQ ID NO: 73 - protein, 372 aa, synthetic construct
DVQLQESGGGLVQPGGSLRLSCAASGFTLDYYAIGWFRQAPGKEREGVSCISGRSDSTNYADSVKGRFTISRDNAKNAVYLQMNSLKPEDTAVYYCAVSGWAGNGCPPIYEYDYWGQGTQVTVSSGGGGSGGGGSGGGGSSRVQPTESIVRFPNITNLCPFGEVFNATRFASVYAWNRKRISNCVADYSVLYNSASFSTFKCYGVSPTKLNDLCFTNVYADSFVIRGDEVRQIAPGQTGKIADYNYKLPDDFTGCVIAWNSNNLDSKVGGNYNYLYRLFRKSNLKPFERDISTEIYQAGSTPCNGVEGFNCYFPLQSYGFQPTNGVGYQPYRVVVLSFELLHAPATVCGPKKSTNLVKNKCVNFHHHHHHHH

SEQ ID NO: 74 - protein, 373 aa, synthetic construct
DVQLQESGGGLVQPGGSLRLSCAASTFTLDYYAIGWFRQAPGKEREGVSCISSRGGSTDYADSVKGRFTISRDNAKNTVYLQMSSLQPEDTAVYYCAAAGWAGYGCPPNRYEYDYWGQGTQVTVSSGGGGSGGGGSGGGGSSRVQPTESIVRFPNITNLCPFGEVFNATRFASVYAWNRKRISNCVADYSVLYNSASFSTFKCYGVSPTKLNDLCFTNVYADSFVIRGDEVRQIAPGQTGKIADYNYKLPDDFTGCVIAWNSNNLDSKVGGNYNYLYRLFRKSNLKPFERDISTEIYQAGSTPCNGVEGFNCYFPLQSYGFQPTNGVGYQPYRVVVLSFELLHAPATVCGPKKSTNLVKNKCVNFHHHHHHHH

SEQ ID NO: 75 - protein, 373 aa, synthetic construct
DVQLQESGGGLVQPGGSLRLSCAASGFTLDYYAIGWFRQAPGEVREEVSCISGRGDSTNYAHSMKGRFTISRDNAKNTVYLQINSLKPEDTAVYYCAAAGWAGYECPANRYEYDYWGQGTQVTVSSGGGGSGGGGSGGGGSSRVQPTESIVRFPNITNLCPFGEVFNATRFASVYAWNRKRISNCVADYSVLYNSASFSTFKCYGVSPTKLNDLCFTNVYADSFVIRGDEVRQIAPGQTGKIADYNYKLPDDFTGCVIAWNSNNLDSKVGGNYNYLYRLFRKSNLKPFERDISTEIYQAGSTPCNGVEGFNCYFPLQSYGFQPTNGVGYQPYRVVVLSFELLHAPATVCGPKKSTNLVKNKCVNFHHHHHHHH

SEQ ID NO: 76 - protein, 373 aa, synthetic construct
DVQLQESGGGLVQPGGSLRLSCAASGFTLDYYAIGWFRQAPGKEREEVSCISSRGGSTNYPDSVKGRFTISRDNAKNTVYLQMNSLRPEDTAVYYCAAAGWAGFGCPPNRYEYDYWGQGTQVTVSSGGGGSGGGGSGGGGSSRVQPTESIVRFPNITNLCPFGEVFNATRFASVYAWNRKRISNCVADYSVLYNSASFSTFKCYGVSPTKLNDLCFTNVYADSFVIRGDEVRQIAPGQTGKIADYNYKLPDDFTGCVIAWNSNNLDSKVGGNYNYLYRLFRKSNLKPFERDISTEIYQAGSTPCNGVEGFNCYFPLQSYGFQPTNGVGYQPYRVVVLSFELLHAPATVCGPKKSTNLVKNKCVNFHHHHHHHH

SEQ ID NO: 77 - protein, 373 aa, synthetic construct
DVQLQESGGGLVQPGGSLRLSCAASGFTLDYYAIGWFRQAPGKEREEVSCISGRGSSTNYADSVKGRFTVSRDNAKNTVYLQINSLKPEDTAVYYCAAAGWAGYGCPANRYEYDYWGQGTQVTVSSGGGGSGGGGSGGGGSSRVQPTESIVRFPNITNLCPFGEVFNATRFASVYAWNRKRISNCVADYSVLYNSASFSTFKCYGVSPTKLNDLCFTNVYADSFVIRGDEVRQIAPGQTGKIADYNYKLPDDFTGCVIAWNSNNLDSKVGGNYNYLYRLFRKSNLKPFERDISTEIYQAGSTPCNGVEGFNCYFPLQSYGFQPTNGVGYQPYRVVVLSFELLHAPATVCGPKKSTNLVKNKCVNFHHHHHHHH

SEQ ID NO: 78 - protein, 373 aa, synthetic construct
DVQLQESGGGLVQPGGSLRLSCAASGFTLDYYAIGWFRQAPGKEREGVSCISSRGGSTNTPDSVKGRFTISRDNAKNTVYLQMNSLRPEDTAVYYCAAAGWAGFGCPPNRYEYDYWGQGTQVTVSSGGGGSGGGGSGGGGSSRVQPTESIVRFPNITNLCPFGEVFNATRFASVYAWNRKRISNCVADYSVLYNSASFSTFKCYGVSPTKLNDLCFTNVYADSFVIRGDEVRQIAPGQTGKIADYNYKLPDDFTGCVIAWNSNNLDSKVGGNYNYLYRLFRKSNLKPFERDISTEIYQAGSTPCNGVEGFNCYFPLQSYGFQPTNGVGYQPYRVVVLSFELLHAPATVCGPKKSTNLVKNKCVNFHHHHHHHH

SEQ ID NO: 79 - protein, 362 aa, synthetic construct
DVQLQESGGGLVQPGGSLRLSCAASGFTLSRSTMTWGRQAPGKGLEWVSDIYRSGSTTYADSVKGRFTISRDDAKNTVYLQMNSLKPEDTAVYYCAVVLPGREYRGQGTQVTVSSGGGGSGGGGSGGGGSSRVQPTESIVRFPNITNLCPFGEVFNATRFASVYAWNRKRISNCVADYSVLYNSASFSTFKCYGVSPTKLNDLCFTNVYADSFVIRGDEVRQIAPGQTGKIADYNYKLPDDFTGCVIAWNSNNLDSKVGGNYNYLYRLFRKSNLKPFERDISTEIYQAGSTPCNGVEGFNCYFPLQSYGFQPTNGVGYQPYRVVVLSFELLHAPATVCGPKKSTNLVKNKCVNFHHHHHHHH

SEQ ID NO: 80 - protein, 754 aa, synthetic construct
DVQLQESGGGLVQPGGSLRLSCAASGFTLSRSTMTWGRQAPGKGLEWVSDIYSSGSTTYADSVKGRFTISRDNAKNTVYLQMNSLKPEDTAVYYCAVVLPGREYRGQGTQVTVSSGGGGSGGGGSGGGGSAENLAVGIGAVFLGFLGAAGSTMGAASMTLTVQARNLLSGIVQQQSNLLRAPEAQQHLLKLTVWGIKQLQARVLAVERYLRDQQLLGIWGCSGKLICTTNVPNLWVTVYYGVPVWKDAETTLFCASDAKAYETEKHNVWATHACVPTDPNPQEIHLENVTEEFNMWKNNMVEQMHTDIISLWDQSLKPCVKLTPLCVTLQCTNVTNNITDDMRGELKNCSFNMTTELRDKKQKVYSLFYRLDVVQINENQGNRSNNSNKEYRLINCNTSAITQACPKVSFEPIPIHYCAPAGFAILKCKDKKFNGTGPCPSVSTVQCTHGIKPVVSTQLLLNGSLAEEEVMIRSENITNNAKNILVQFNTPVQINCTRPNNNTRKSIRIGPGQAFYATGDIIGDIRQAHCNVSKATWNETLGKVVKQLRKHFGNNTIIRFANSSGGDLEVTTHSFNCGGEFFYCNTSGLFNSTWISNTSVQGSNSTGSNDSITLPCRIKQIINMWQRIGQAMYAPPIQGVIRCVSNITGLILTRDGGSTNSTTETFRPGGGDMRDNWRSELYKYKVVKIEPLGVAPTRRNLSEIWDNMTWLQWDKEISNYTQIIYGLLEESQNQQEKNEQDLLALDHHHHHHHH

SEQ ID NO: 81 - protein, 765 aa, synthetic construct
DVQLQESGGGLVQPGGSLRLSCAASTFTLDYYAIGWFRQAPGKEREGVSCISSRGGSTDYADSVKGRFTISRDNAKNTVYLQMSSLQPEDTAVYYCAAAGWAGYGCPPNRYEYDYWGQGTQVTVSSGGGGSGGGGSGGGGSAENLAVGIGAVFLGFLGAAGSTMGAASMTLTVQARNLLSGIVQQQSNLLRAPEAQQHLLKLTVWGIKQLQARVLAVERYLRDQQLLGIWGCSGKLICTTNVPNLWVTVYYGVPVWKDAETTLFCASDAKAYETEKHNVWATHACVPTDPNPQEIHLENVTEEFNMWKNNMVEQMHTDIISLWDQSLKPCVKLTPLCVTLQCTNVTNNITDDMRGELKNCSFNMTTELRDKKQKVYSLFYRLDVVQINENQGNRSNNSNKEYRLINCNTSAITQACPKVSFEPIPIHYCAPAGFAILKCKDKKFNGTGPCPSVSTVQCTHGIKPVVSTQLLLNGSLAEEEVMIRSENITNNAKNILVQFNTPVQINCTRPNNNTRKSIRIGPGQAFYATGDIIGDIRQAHCNVSKATWNETLGKVVKQLRKHFGNNTIIRFANSSGGDLEVTTHSFNCGGEFFYCNTSGLFNSTWISNTSVQGSNSTGSNDSITLPCRIKQIINMWQRIGQAMYAPPIQGVIRCVSNITGLILTRDGGSTNSTTETFRPGGGDMRDNWRSELYKYKVVKIEPLGVAPTRRNLSEIWDNMTWLQWDKEISNYTQIIYGLLEESQNQQEKNEQDLLALDHHHHHHHH

SEQ ID NO: 82 - protein, 764 aa, synthetic construct
DVQLQESGGGLVQPGGSLRLSCAASGFTLDYYAIGWFRQAPGKEREGVSCISGRSDSTNYADSVKGRFTISRDNAKNAVYLQMNSLKPEDTAVYYCAVSGWAGNGCPPIYEYDYWGQGTQVTVSSGGGGSGGGGSGGGGSAENLAVGIGAVFLGFLGAAGSTMGAASMTLTVQARNLLSGIVQQQSNLLRAPEAQQHLLKLTVWGIKQLQARVLAVERYLRDQQLLGIWGCSGKLICTTNVPNLWVTVYYGVPVWKDAETTLFCASDAKAYETEKHNVWATHACVPTDPNPQEIHLENVTEEFNMWKNNMVEQMHTDIISLWDQSLKPCVKLTPLCVTLQCTNVTNNITDDMRGELKNCSFNMTTELRDKKQKVYSLFYRLDVVQINENQGNRSNNSNKEYRLINCNTSAITQACPKVSFEPIPIHYCAPAGFAILKCKDKKFNGTGPCPSVSTVQCTHGIKPVVSTQLLLNGSLAEEEVMIRSENITNNAKNILVQFNTPVQINCTRPNNNTRKSIRIGPGQAFYATGDIIGDIRQAHCNVSKATWNETLGKVVKQLRKHFGNNTIIRFANSSGGDLEVTTHSFNCGGEFFYCNTSGLFNSTWISNTSVQGSNSTGSNDSITLPCRIKQIINMWQRIGQAMYAPPIQGVIRCVSNITGLILTRDGGSTNSTTETFRPGGGDMRDNWRSELYKYKVVKIEPLGVAPTRRNLSEIWDNMTWLQWDKEISNYTQIIYGLLEESQNQQEKNEQDLLALDHHHHHHHH

SEQ ID NO: 83 - protein, 765 aa, synthetic construct; identical to SEQ ID NO: 36

SEQ ID NO: 84 - protein, 765 aa, synthetic construct
DVQLQESGGGLVQPGGSLRLSCAASGFTLDYYAIGWFRQAPGKEREEVSCISSRGGSTNYPDSVKGRFTISRDNAKNTVYLQMNSLRPEDTAVYYCAAAGWAGFGCPPNRYEYDYWGQGTQVTVSSGGGGSGGGGSGGGGSAENLAVGIGAVFLGFLGAAGSTMGAASMTLTVQARNLLSGIVQQQSNLLRAPEAQQHLLKLTVWGIKQLQARVLAVERYLRDQQLLGIWGCSGKLICTTNVPNLWVTVYYGVPVWKDAETTLFCASDAKAYETEKHNVWATHACVPTDPNPQEIHLENVTEEFNMWKNNMVEQMHTDIISLWDQSLKPCVKLTPLCVTLQCTNVTNNITDDMRGELKNCSFNMTTELRDKKQKVYSLFYRLDVVQINENQGNRSNNSNKEYRLINCNTSAITQACPKVSFEPIPIHYCAPAGFAILKCKDKKFNGTGPCPSVSTVQCTHGIKPVVSTQLLLNGSLAEEEVMIRSENITNNAKNILVQFNTPVQINCTRPNNNTRKSIRIGPGQAFYATGDIIGDIRQAHCNVSKATWNETLGKVVKQLRKHFGNNTIIRFANSSGGDLEVTTHSFNCGGEFFYCNTSGLFNSTWISNTSVQGSNSTGSNDSITLPCRIKQIINMWQRIGQAMYAPPIQGVIRCVSNITGLILTRDGGSTNSTTETFRPGGGDMRDNWRSELYKYKVVKIEPLGVAPTRRNLSEIWDNMTWLQWDKEISNYTQIIYGLLEESQNQQEKNEQDLLALDHHHHHHHH

SEQ ID NO: 85 - protein, 765 aa, synthetic construct
DVQLQESGGGLVQPGGSLRLSCAASGFTLDYYAIGWFRQAPGEVREEVSCISGRGDSTNYAHSMKGRFTISRDNAKNTVYLQINSLKPEDTAVYYCAAAGWAGYECPANRYEYDYWGQGTQVTVSSGGGGSGGGGSGGGGSAENLAVGIGAVFLGFLGAAGSTMGAASMTLTVQARNLLSGIVQQQSNLLRAPEAQQHLLKLTVWGIKQLQARVLAVERYLRDQQLLGIWGCSGKLICTTNVPNLWVTVYYGVPVWKDAETTLFCASDAKAYETEKHNVWATHACVPTDPNPQEIHLENVTEEFNMWKNNMVEQMHTDIISLWDQSLKPCVKLTPLCVTLQCTNVTNNITDDMRGELKNCSFNMTTELRDKKQKVYSLFYRLDVVQINENQGNRSNNSNKEYRLINCNTSAITQACPKVSFEPIPIHYCAPAGFAILKCKDKKFNGTGPCPSVSTVQCTHGIKPVVSTQLLLNGSLAEEEVMIRSENITNNAKNILVQFNTPVQINCTRPNNNTRKSIRIGPGQAFYATGDIIGDIRQAHCNVSKATWNETLGKVVKQLRKHFGNNTIIRFANSSGGDLEVTTHSFNCGGEFFYCNTSGLFNSTWISNTSVQGSNSTGSNDSITLPCRIKQIINMWQRIGQAMYAPPIQGVIRCVSNITGLILTRDGGSTNSTTETFRPGGGDMRDNWRSELYKYKVVKIEPLGVAPTRRNLSEIWDNMTWLQWDKEISNYTQIIYGLLEESQNQQEKNEQDLLALDHHHHHHHH

SEQ ID NO: 86 - protein, 765 aa, synthetic construct
DVQLQESGGGLVQPGGSTRLSCAASGFTLDYYAIGWFRQAPGKEREEVSCMSSRGGSTNYVDSVQGRFTLSRDNAKNTVYLQMNSLKPEDTAVYYCAAAGWAGNGCPPNRYEYDYWGQGTQVTVSSGGGGSGGGGSGGGGSAENLAVGIGAVFLGFLGAAGSTMGAASMTLTVQARNLLSGIVQQQSNLLRAPEAQQHLLKLTVWGIKQLQARVLAVERYLRDQQLLGIWGCSGKLICTTNVPNLWVTVYYGVPVWKDAETTLFCASDAKAYETEKHNVWATHACVPTDPNPQEIHLENVTEEFNMWKNNMVEQMHTDIISLWDQSLKPCVKLTPLCVTLQCTNVTNNITDDMRGELKNCSFNMTTELRDKKQKVYSLFYRLDVVQINENQGNRSNNSNKEYRLINCNTSAITQACPKVSFEPIPIHYCAPAGFAILKCKDKKFNGTGPCPSVSTVQCTHGIKPVVSTQLLLNGSLAEEEVMIRSENITNNAKNILVQFNTPVQINCTRPNNNTRKSIRIGPGQAFYATGDIIGDIRQAHCNVSKATWNETLGKVVKQLRKHFGNNTIIRFANSSGGDLEVTTHSFNCGGEFFYCNTSGLFNSTWISNTSVQGSNSTGSNDSITLPCRIKQIINMWQRIGQAMYAPPIQGVIRCVSNITGLILTRDGGSTNSTTETFRPGGGDMRDNWRSELYKYKVVKIEPLGVAPTRRNLSEIWDNMTWLQWDKEISNYTQIIYGLLEESQNQQEKNEQDLLALDHHHHHHHH

SEQ ID NO: 87 - protein, 765 aa, synthetic construct
DVQLQESGGGLVQPGGSLRLSCAASRFTLDYYAIGWFRQAPGKEREEVSCISSRAGSTNYQDSVKGRFTISRDNAKNTVYLQMNSLKPEDTAVYYCAAAGWAGNACPPNRYEYDYWGQGTQVTVSSGGGGSGGGGSGGGGSAENLAVGIGAVFLGFLGAAGSTMGAASMTLTVQARNLLSGIVQQQSNLLRAPEAQQHLLKLTVWGIKQLQARVLAVERYLRDQQLLGIWGCSGKLICTTNVPNLWVTVYYGVPVWKDAETTLFCASDAKAYETEKHNVWATHACVPTDPNPQEIHLENVTEEFNMWKNNMVEQMHTDIISLWDQSLKPCVKLTPLCVTLQCTNVTNNITDDMRGELKNCSFNMTTELRDKKQKVYSLFYRLDVVQINENQGNRSNNSNKEYRLINCNTSAITQACPKVSFEPIPIHYCAPAGFAILKCKDKKFNGTGPCPSVSTVQCTHGIKPVVSTQLLLNGSLAEEEVMIRSENITNNAKNILVQFNTPVQINCTRPNNNTRKSIRIGPGQAFYATGDIIGDIRQAHCNVSKATWNETLGKVVKQLRKHFGNNTIIRFANSSGGDLEVTTHSFNCGGEFFYCNTSGLFNSTWISNTSVQGSNSTGSNDSITLPCRIKQIINMWQRIGQAMYAPPIQGVIRCVSNITGLILTRDGGSTNSTTETFRPGGGDMRDNWRSELYKYKVVKIEPLGVAPTRRNLSEIWDNMTWLQWDKEISNYTQIIYGLLEESQNQQEKNEQDLLALDHHHHHHHH

SEQ ID NO: 88 - protein, 122 aa, synthetic construct
DVQLQESGGGLVKPGGSLTLSCAASRSIFTINTMGWYRQAPGKQRELVADITNGGGRNYADSVKGRFTIGRDNAKNTVYLTMNSLKPEDTAVYYCNARVLVWPSPPDDYWGQGTQVTVSSGR

SEQ ID NO: 89 - protein, 780 aa, synthetic construct
MGWSCIILFLVATATGVHSDVQLQESGGGLVKPGGSLTLSCAASRSIFTINTMGWYRQAPGKQRELVADITNGGGRNYADSVKGRFTIGRDNAKNTVYLTMNSLKPEDTAVYYCNARVLVWPSPPDDYWGQGTQVTVSSGRGGGGSGGGGSGGGGSAENLAVGIGAVFLGFLGAAGSTMGAASMTLTVQARNLLSGIVQQQSNLLRAPEAQQHLLKLTVWGIKQLQARVLAVERYLRDQQLLGIWGCSGKLICTTNVPNLWVTVYYGVPVWKDAETTLFCASDAKAYETEKHNVWATHACVPTDPNPQEIHLENVTEEFNMWKNNMVEQMHTDIISLWDQSLKPCVKLTPLCVTLQCTNVTNNITDDMRGELKNCSFNMTTELRDKKQKVYSLFYRLDVVQINENQGNRSNNSNKEYRLINCNTSAITQACPKVSFEPIPIHYCAPAGFAILKCKDKKFNGTGPCPSVSTVQCTHGIKPVVSTQLLLNGSLAEEEVMIRSENITNNAKNILVQFNTPVQINCTRPNNNTRKSIRIGPGQAFYATGDIIGDIRQAHCNVSKATWNETLGKVVKQLRKHFGNNTIIRFANSSGGDLEVTTHSFNCGGEFFYCNTSGLFNSTWISNTSVQGSNSTGSNDSITLPCRIKQIINMWQRIGQAMYAPPIQGVIRCVSNITGLILTRDGGSTNSTTETFRPGGGDMRDNWRSELYKYKVVKIEPLGVAPTRRNLSEIWDNMTWLQWDKEISNYTQIIYGLLEESQNQQEKNEQDLLALDHHHHHHHH

SEQ ID NO: 90 - protein, 8 aa, synthetic construct
GFTLSRST

SEQ ID NO: 91 - protein, 7 aa, synthetic construct
IYSSGST

SEQ ID NO: 92 - protein, 12 aa, synthetic construct
AVVLPGREYRGQ

SEQ ID NO: 93 - protein, 8 aa, synthetic construct
GFSLDYYA

SEQ ID NO: 94 - protein, 8 aa, synthetic construct
VSGREGST

SEQ ID NO: 95 - protein, 19 aa, synthetic construct
AAAGWNGLGCPPSLYEYDY

SEQ ID NO: 96 - protein, 8 aa, synthetic construct
GFTLDEYT

SEQ ID NO: 97 - protein, 8 aa, synthetic construct
ISSRGGRT

SEQ ID NO: 98 - protein, 17 aa, synthetic construct
AAASYYDDCRVPAWYDY

SEQ ID NO: 99 - protein, 8 aa, synthetic construct
GFTLDYYT

SEQ ID NO: 100 - protein, 8 aa, synthetic construct
ISSSDDST

SEQ ID NO: 101 - protein, 24 aa, synthetic construct
AAVPRHTGISPVLAMCASSVWYDY

SEQ ID NO: 102 - protein, 8 aa, synthetic construct
GFTLDYYA

SEQ ID NO: 103 - protein, 8 aa, synthetic construct
LSGRNGSP

SEQ ID NO: 104 - protein, 19 aa, synthetic construct
AAAGWNGLGCPPSLYEYDY

SEQ ID NO: 105 - protein, 8 aa, synthetic construct
GFTLDYYA

SEQ ID NO: 106 - protein, 8 aa, synthetic construct
ISGRSDST

SEQ ID NO: 107 - protein, 18 aa, synthetic construct
AVSGWAGNGCPPIYEYDY

SEQ ID NO: 108 - protein, 8 aa, synthetic construct
GFTLDYYA

SEQ ID NO: 109 - protein, 8 aa, synthetic construct
ISSRGGST

SEQ ID NO: 110 - protein, 19 aa, synthetic construct
AAAGWAGFGCPPNRYEYDY

SEQ ID NO: 111 - protein, 8 aa, synthetic construct
GFTLDYYA

SEQ ID NO: 112 - protein, 8 aa, synthetic construct
ISGRGGST

SEQ ID NO: 113 - protein, 19 aa, synthetic construct
AAAGWAGNVCPPNRYEYDY

SEQ ID NO: 114 - protein, 8 aa, synthetic construct
GFTLDYYA

SEQ ID NO: 115 - protein, 8 aa, synthetic construct
ISGRGDST

SEQ ID NO: 116 - protein, 19 aa, synthetic construct
AAAGWAGNVCPPNRYEYDY

SEQ ID NO: 117 - protein, 8 aa, synthetic construct
GFTLDYYA

SEQ ID NO: 118 - protein, 8 aa, synthetic construct
ISGRGSST

SEQ ID NO: 119 - protein, 19 aa, synthetic construct
AAAGWAGYGCPANRYEYDY

SEQ ID NO: 120 - protein, 8 aa, synthetic construct
GFTLDYYA

SEQ ID NO: 121 - protein, 8 aa, synthetic construct
MSSRGGST

SEQ ID NO: 122 - protein, 19 aa, synthetic construct
AAAGWAGNGCPPNRYEYDY

SEQ ID NO: 123 - protein, 8 aa, synthetic construct
GFTLSRST

SEQ ID NO: 124 - protein, 7 aa, synthetic construct
IYRSGST

SEQ ID NO: 125 - protein, 11 aa, synthetic construct
VVLPGREYRGQ

SEQ ID NO: 126 - protein, 8 aa, synthetic construct
TFTLDYYA

SEQ ID NO: 127 - protein, 8 aa, synthetic construct
ISSRSGST

SEQ ID NO: 128 - protein, 19 aa, synthetic construct
AAAGWAGYGCPANRYEYDY

SEQ ID NO: 129 - protein, 8 aa, synthetic construct
GFTLDHYA

SEQ ID NO: 130 - protein, 8 aa, synthetic construct
ISSRRGST

SEQ ID NO: 131 - protein, 19 aa, synthetic construct
AAAGWAGYMCPPNRYEYDY

SEQ ID NO: 132 - protein, 8 aa, synthetic construct
RFTLDYYA

SEQ ID NO: 133 - protein, 8 aa, synthetic construct
ISSRAGST

SEQ ID NO: 134 - protein, 19 aa, synthetic construct
AAAGWAGNACPPNRYEYDY

SEQ ID NO: 135 - protein, 8 aa, synthetic construct
GFTLDYYA

SEQ ID NO: 136 - protein, 8 aa, synthetic construct
ISGRRGST

SEQ ID NO: 137 - protein, 19 aa, synthetic construct
AAAGWNGLGCPPSLDEYDY

SEQ ID NO: 138 - protein, 8 aa, synthetic construct
GFTLDYYA

SEQ ID NO: 139 - protein, 8 aa, synthetic construct
VSGRHGST

SEQ ID NO: 140 - protein, 19 aa, synthetic construct
AAAGWNGLGCPPSLDEYDY

SEQ ID NO: 141 - protein, 8 aa, synthetic construct
GLTLDYYN

SEQ ID NO: 142 - protein, 8 aa, synthetic construct
ISVSGGVT

SEQ ID NO: 143 - protein, 19 aa, synthetic construct
AAVSLPFVPMLGCPEGYDY